European Patent Application EP 4 242 232 A1, published September 13, 2023. Title: BISPECIFIC ANTIBODY AND USE THEREOF. Applicant: Bio-Thera Solutions, Ltd. Application EP21888662.0. The sequence listing filed with the application follows.

SEQUENCE LISTING (102 sequences)

SEQ ID NO: 1 - protein, 139 aa, Artificial Sequence
  synthetic construct
MWPLVAALLLGSACCGSAQLLFNKTKSVEFTFCNDTVVIPCFVTNMEAQNTTEVYVKWKFKGRDIYTFDGALNKSTVPTDFSSAKIEVSQLLKGDASLKMDKSDAVSHTGNYTCEVTELTREGETIIELKYRVVSWFSP

SEQ ID NO: 2 - protein, 238 aa, Artificial Sequence
  synthetic construct
MRIFAVFIFMTYWHLLNAFTVTVPKDLYVVEYGSNMTIECKFPVEKQLDLAALIVYWEMEDKNIIQFVHGEEDLKVQHSSYRQRARLLKDQLSLGNAALQITDVKLQDAGVYRCMISYGGADYKRITVKVNAPYNKINQRILVVDPVTSEHELTCQAEGYPKAEVIWTSSDHQVLSGKTTTTNSKREEKLFNVTSTLRINTTTNEIFYCTFRRLDPEENHTAELVIPELPLAHPPNER

SEQ ID NO: 3 - protein, 8 aa, Artificial Sequence
  synthetic construct
HHHHHHHH

SEQ ID NO: 4 - protein, 10 aa, Artificial Sequence
  synthetic construct
GFTFSDSWIH

SEQ ID NO: 5 - protein, 10 aa, Artificial Sequence
  synthetic construct
SFSLKDSWIH

SEQ ID NO: 6 - protein, 10 aa, Artificial Sequence
  synthetic construct
GWATRDSWIH

SEQ ID NO: 7 - protein, 10 aa, Artificial Sequence
  synthetic construct
NSHLRDSWIH

SEQ ID NO: 8 - protein, 10 aa, Artificial Sequence
  synthetic construct
GLRPADSWIH

SEQ ID NO: 9 - protein, 18 aa, Artificial Sequence
  synthetic construct
GWISPYGGSTYYADSVKG

SEQ ID NO: 10 - protein, 18 aa, Artificial Sequence
  synthetic construct
GWISPYGGSTYYADDFRH

SEQ ID NO: 11 - protein, 18 aa, Artificial Sequence
  synthetic construct
GWISPYGGSTYYADSLGD

SEQ ID NO: 12 - protein, 18 aa, Artificial Sequence
  synthetic construct
GWISPYGGSTYYADHLSQ

SEQ ID NO: 13 - protein, 18 aa, Artificial Sequence
  synthetic construct
GWISPYGGSTYYADGMRS

SEQ ID NO: 14 - protein, 18 aa, Artificial Sequence
  synthetic construct
GWISPYGGSTYYADSYRS

SEQ ID NO: 15 - protein, 18 aa, Artificial Sequence
  synthetic construct
GWISPYGGSTYYADPYVG

SEQ ID NO: 16 - protein, 18 aa, Artificial Sequence
  synthetic construct
GWISPYGGSTYYADSLKG

SEQ ID NO: 17 - protein, 18 aa, Artificial Sequence
  synthetic construct
GWISPYGGSTYYADSYRA

SEQ ID NO: 18 - protein, 18 aa, Artificial Sequence
  synthetic construct
GWISPYGGSTYYADYLHG

SEQ ID NO: 19 - protein, 9 aa, Artificial Sequence
  synthetic construct
RHWPGGFDY

SEQ ID NO: 20 - protein, 9 aa, Artificial Sequence
  synthetic construct
RHWPGGLLP

SEQ ID NO: 21 - protein, 6 aa, Artificial Sequence
  synthetic construct
DNYYWS

SEQ ID NO: 22 - protein, 6 aa, Artificial Sequence
  synthetic construct
DGYYWS

SEQ ID NO: 23 - protein, 6 aa, Artificial Sequence
  synthetic construct
NDYYWS

SEQ ID NO: 24 - protein, 16 aa, Artificial Sequence
  synthetic construct
YIYYSGNTNYNPSLKS

SEQ ID NO: 25 - protein, 16 aa, Artificial Sequence
  synthetic construct
RIYGNSTTNYNPSLKS

SEQ ID NO: 26 - protein, 16 aa, Artificial Sequence
  synthetic construct
RIYGNGDTNYNPSLKS

SEQ ID NO: 27 - protein, 16 aa, Artificial Sequence
  synthetic construct
RIYYNGNTNYNPSLKS

SEQ ID NO: 28 - protein, 16 aa, Artificial Sequence
  synthetic construct
RIYGDSATNYNPSLKS

SEQ ID NO: 29 - protein, 8 aa, Artificial Sequence
  synthetic construct
GGRFLERY

SEQ ID NO: 30 - protein, 8 aa, Artificial Sequence
  synthetic construct
GGRIFGGY

SEQ ID NO: 31 - protein, 8 aa, Artificial Sequence
  synthetic construct
GGRIFAGY

SEQ ID NO: 32 - protein, 8 aa, Artificial Sequence
  synthetic construct
GGRILAGY

SEQ ID NO: 33 - protein, 8 aa, Artificial Sequence
  synthetic construct
GGRIFSGY

SEQ ID NO: 34 - protein, 7 aa, Artificial Sequence
  synthetic construct
GRGIFGY

SEQ ID NO: 35 - protein, 7 aa, Artificial Sequence
  synthetic construct
GGRIFGH

SEQ ID NO: 36 - protein, 11 aa, Artificial Sequence
  synthetic construct
LASQTIGTWLA

SEQ ID NO: 37 - protein, 11 aa, Artificial Sequence
  synthetic construct
QASQDIGKHLN

SEQ ID NO: 38 - protein, 11 aa, Artificial Sequence
  synthetic construct
RASQGIGSWLA

SEQ ID NO: 39 - protein, 11 aa, Artificial Sequence
  synthetic construct
RASQGISSYLA

SEQ ID NO: 40 - protein, 11 aa, Artificial Sequence
  synthetic construct
RASQGIGKFLA

SEQ ID NO: 41 - protein, 7 aa, Artificial Sequence
  synthetic construct
AASTLQS

SEQ ID NO: 42 - protein, 7 aa, Artificial Sequence
  synthetic construct
GASNLKT

SEQ ID NO: 43 - protein, 7 aa, Artificial Sequence
  synthetic construct
AASSLQS

SEQ ID NO: 44 - protein, 7 aa, Artificial Sequence
  synthetic construct
AASRLQS

SEQ ID NO: 45 - protein, 9 aa, Artificial Sequence
  synthetic construct
QQYYSTPRT

SEQ ID NO: 46 - protein, 9 aa, Artificial Sequence
  synthetic construct
QQSYTTPYT

SEQ ID NO: 47 - protein, 9 aa, Artificial Sequence
  synthetic construct
QQYFSTPYT

SEQ ID NO: 48 - protein, 9 aa, Artificial Sequence
  synthetic construct
QQYYSTPYT

SEQ ID NO: 49 - protein, 118 aa, Artificial Sequence
  synthetic construct
EVQLVESGGGLVQPGGSLRLSCAASGFTFSDSWIHWVRQAPGKGLEWVGWISPYGGSTYYADSVKGRFTISADTSKNTAYLQMNSLRAEDTAVYYCARRHWPGGFDYWGQGTLVTVSS

SEQ ID NO: 50 - protein, 118 aa, Artificial Sequence
  synthetic construct
EVQLVESGGGLVQPGGSLRLSCAASGFTFSDSWIHWVRQAPGKGLEWVGWISPYGGSTYYADDFRHRFTISADTSKNTAYLQMNSLRAEDTAVYYCARRHWPGGFDYWGQGTLVTVSS

SEQ ID NO: 51 - protein, 118 aa, Artificial Sequence
  synthetic construct
EVQLVESGGGLVQPGGSLRLSCAASGFTFSDSWIHWVRQAPGKGLEWVGWISPYGGSTYYADSLGDRFTISADTSKNTAYLQMNSLRAEDTAVYYCARRHWPGGFDYWGQGTLVTVSS

SEQ ID NO: 52 - protein, 118 aa, Artificial Sequence
  synthetic construct
EVQLVESGGGLVQPGGSLRLSCAASGFTFSDSWIHWVRQAPGKGLEWVGWISPYGGSTYYADHLSQRFTISADTSKNTAYLQMNSLRAEDTAVYYCARRHWPGGFDYWGQGTLVTVSS

SEQ ID NO: 53 - protein, 118 aa, Artificial Sequence
  synthetic construct
EVQLVESGGGLVQPGGSLRLSCAASGFTFSDSWIHWVRQAPGKGLEWVGWISPYGGSTYYADGMRSRFTISADTSKNTAYLQMNSLRAEDTAVYYCARRHWPGGFDYWGQGTLVTVSS

SEQ ID NO: 54 - protein, 118 aa, Artificial Sequence
  synthetic construct
EVQLVESGGGLVQPGGSLRLSCAASGFTFSDSWIHWVRQAPGKGLEWVGWISPYGGSTYYADSYRSRFTISADTSKNTAYLQMNSLRAEDTAVYYCARRHWPGGFDYWGQGTLVTVSS

SEQ ID NO: 55 - protein, 118 aa, Artificial Sequence
  synthetic construct
EVQLVESGGGLVQPGGSLRLSCAASGFTFSDSWIHWVRQAPGKGLEWVGWISPYGGSTYYADPYVGRFTISADTSKNTAYLQMNSLRAEDTAVYYCARRHWPGGFDYWGQGTLVTVSS

SEQ ID NO: 56 - protein, 118 aa, Artificial Sequence
  synthetic construct
EVQLVESGGGLVQPGGSLRLSCAASGFTFSDSWIHWVRQAPGKGLEWVGWISPYGGSTYYADSLKGRFTISADTSKNTAYLQMNSLRAEDTAVYYCARRHWPGGFDYWGQGTLVTVSS

SEQ ID NO: 57 - protein, 118 aa, Artificial Sequence
  synthetic construct
EVQLVESGGGLVQPGGSLRLSCAASGFTFSDSWIHWVRQAPGKGLEWVGWISPYGGSTYYADSYRARFTISADTSKNTAYLQMNSLRAEDTAVYYCARRHWPGGFDYWGQGTLVTVSS

SEQ ID NO: 58 - protein, 118 aa, Artificial Sequence
  synthetic construct
EVQLVESGGGLVQPGGSLRLSCAASGFTFSDSWIHWVRQAPGKGLEWVGWISPYGGSTYYADYLHGRFTISADTSKNTAYLQMNSLRAEDTAVYYCARRHWPGGFDYWGQGTLVTVSS

SEQ ID NO: 59 - protein, 118 aa, Artificial Sequence
  synthetic construct
EVQLVESGGGLVQPGGSLRLSCAASSFSLKDSWIHWVRQAPGKGLEWVGWISPYGGSTYYADSVKGRFTISADTSKNTAYLQMNSLRAEDTAVYYCARRHWPGGFDYWGQGTLVTVSS

SEQ ID NO: 60 - protein, 118 aa, Artificial Sequence
  synthetic construct
EVQLVESGGGLVQPGGSLRLSCAASGWATRDSWIHWVRQAPGKGLEWVGWISPYGGSTYYADSVKGRFTISADTSKNTAYLQMNSLRAEDTAVYYCARRHWPGGFDYWGQGTLVTVSS

SEQ ID NO: 61 - protein, 118 aa, Artificial Sequence
  synthetic construct
EVQLVESGGGLVQPGGSLRLSCAASGFTFSDSWIHWVRQAPGKGLEWVGWISPYGGSTYYADSVKGRFTISADTSKNTAYLQMNSLRAEDTAVYYCARRHWPGGLLPWGQGTLVTVSS

SEQ ID NO: 62 - protein, 118 aa, Artificial Sequence
  synthetic construct
EVQLVESGGGLVQPGGSLRLSCAASGLRPADSWIHWVRQAPGKGLEWVGWISPYGGSTYYADSVKGRFTISADTSKNTAYLQMNSLRAEDTAVYYCARRHWPGGFDYWGQGTLVTVSS

SEQ ID NO: 63 - protein, 118 aa, Artificial Sequence
  synthetic construct
EVQLVESGGGLVQPGGSLRLSCAASNSHLRDSWIHWVRQAPGKGLEWVGWISPYGGSTYYADSVKGRFTISADTSKNTAYLQMNSLRAEDTAVYYCARRHWPGGFDYWGQGTLVTVSS

SEQ ID NO: 64 - protein, 116 aa, Artificial Sequence
  synthetic construct
QVQLQESGPGLVKPSETLSLTCTVSGGSLDNYYWSWIRQPPGKGLEWIGYIYYSGNTNYNPSLKSRVTISVDTSKNQFSLKLSSVTAADTAVYYCARGGRFLERYWGQGTLVTVSS

SEQ ID NO: 65 - protein, 116 aa, Artificial Sequence
  synthetic construct
QVQLQESGPGLVKPSETLSLTCTVSGGSLDNYYWSWIRQPPGKGLEWIGYIYYSGNTNYNPSLKSRVTISVDTSKNQFSLRLRSVTAADTAVYYCARGGRFLERYWGQGTLVTVSS

SEQ ID NO: 66 - protein, 116 aa, Artificial Sequence
  synthetic construct
QVQLQESGPGLVKPSETLSLTCTVSGGSLDNYYWSWIRQPPGKGLEWIGYIYYSGNTNYNPSLKSRVTISVDTSKNQFSLRLRSVTAADTAVYYCARGGRIFGGYWGQGTLVTVSS

SEQ ID NO: 67 - protein, 116 aa, Artificial Sequence
  synthetic construct
QVQLQESGPGLVKPSETLSLTCTVSGGSLDNYYWSWIRQPPGKGLEWIGYIYYSGNTNYNPSLKSRVTISVDTSKNQFSLRLRSVTAADTAVYYCARGGRIFAGYWGQGTLVTVSS

SEQ ID NO: 68 - protein, 116 aa, Artificial Sequence
  synthetic construct
QVQLQESGPGLVKPSETLSLTCTVSGGSLDGYYWSWIRQPPGKGLEWIGRIYGNSTTNYNPSLKSRVTISVDTSKNQFSLRLRSVTAADTAVYYCARGGRIFAGYWGQGTLVTVSS

SEQ ID NO: 69 - protein, 116 aa, Artificial Sequence
  synthetic construct
QVQLQESGPGLVKPSETLSLTCTVSGGSLNDYYWSWIRQPPGKGLEWIGRIYGNGDTNYNPSLKSRVTISVDTSKNQFSLRLRSVTAADTAVYYCARGGRILAGYWGQGTLVTVSS

SEQ ID NO: 70 - protein, 116 aa, Artificial Sequence
  synthetic construct
QVQLQESGPGLVKPSETLSLTCTVSGGSLDNYYWSWIRQPPGKGLEWIGRIYYNGNTNYNPSLKSRVTISVDTSKNQFSLRLRSVTAADTAVYYCARGGRILAGYWGQGTLVTVSS

SEQ ID NO: 71 - protein, 116 aa, Artificial Sequence
  synthetic construct
QVQLQESGPGLVKPSETLSLTCTVSGGSLDNYYWSWIRQPPGKGLEWIGYIYYSGNTNYNPSLKSRVTISVDTSKNQFSLRLRSVTAADTAVYYCARGGRIFSGYWGQGTLVTVSS

SEQ ID NO: 72 - protein, 115 aa, Artificial Sequence
  synthetic construct
QVQLQESGPGLVKPSETLSLTCTVSGGSLDNYYWSWIRQPPGKGLEWIGYIYYSGNTNYNPSLKSRVTISVDTSKNQFSLRLRSVTAADTAVYYCARGRGIFGYWGQGTLVTVSS

SEQ ID NO: 73 - protein, 116 aa, Artificial Sequence
  synthetic construct
QVQLQESGPGLVKPSETLSLTCTVSGGSLDNYYWSWIRQPPGKGLEWIGRIYGDSATNYNPSLKSRVTISVDTSKNQFSLRLRSVTAADTAVYYCARGGRIFSGYWGQGTLVTVSS

SEQ ID NO: 74 - protein, 115 aa, Artificial Sequence
  synthetic construct
QVQLQESGPGLVKPSETLSLTCTVSGGSLDNYYWSWIRQPPGKGLEWIGYIYYSGNTNYNPSLKSRVTISVDTSKNQFSLRLRSVTAADTAVYYCARGGRIFGHWGQGTLVTVSS

SEQ ID NO: 75 - protein, 107 aa, Artificial Sequence
  synthetic construct
EIVLTQSPSSLSASVGDRVTITCLASQTIGTWLAWYQQKPGKSPQLLIYAASTLQSGVPSRFSGSGSGTDFTLTISSLQPEDVATYYCQQYYSTPRTFGQGTKVEIK

SEQ ID NO: 76 - protein, 107 aa, Artificial Sequence
  synthetic construct
EIVLTQSPSSVSASVGDKLTMTCQASQDIGKHLNWYQQKPGKPPKLLIYGASNLKTGVPSRFSGTGSGTDFTLTISSLQPEDFATYYCQQSYTTPYTFGQGTRLEIK

SEQ ID NO: 77 - protein, 107 aa, Artificial Sequence
  synthetic construct
EIVLTQSPSSVSASVGDRITITCRASQGIGSWLAWYQQKPGKAPSLLIYAASSLQSGVPSRFSGSGSGTDFTLTISSLQTEDVAVYYCQQYFSTPYTFGQGTKVDIK

SEQ ID NO: 78 - protein, 107 aa, Artificial Sequence
  synthetic construct
DIQMTQSPSSFSASTGDRVTITCRASQGISSYLAWYQQKPGKAPKLLIYAASRLQSGVPSRFSGSGSGTDFTLTISSLQAEDVAVYYCQQYYSTPYTFGQGTKVDIK

SEQ ID NO: 79 - protein, 107 aa, Artificial Sequence
  synthetic construct
DIQMTQSPSSLSASVGDRVTIPCRASQGIGKFLAWYQQKPGKAPSLLIYAASSLQSGVPSRFSGSGSGTDFTLTISSLQTEDVAVYYCQQYFSTPYTFGQGTKVDIK

SEQ ID NO: 80 - protein, 107 aa, Artificial Sequence
  synthetic construct
DIQMTQSPSSLSASVGDRVTITCLASQTIGTWLAWYQQKPGKSPQLLIYAASSLQSGVPSRFSGSGSGTDFTLTISSLQPEDVATYYCQQYYSTPYTFGQGTKVDIK

SEQ ID NO: 81 - protein, 330 aa, Artificial Sequence [sequence omitted]

SEQ ID NO: 82 - protein, 107 aa, Artificial Sequence [sequence omitted]

SEQ ID NO: 83 - protein, 330 aa, Artificial Sequence
  synthetic construct
ASTKGPSVFPLAPSSKSTSGGTAALGCLVKDYFPEPVTVSWNSGALTSGVHTFPAVLQSSGLYSLSSVVTVPSSSLGTQTYICNVNHKPSNTKVDKKVEPKSCDKTHTCPPCPAPELLGGPSVFLFPPKPKDTLMISRTPEVTCVVVDVSHEDPEVKFNWYVDGVEVHNAKTKPREEQYNSTYRVVSVLTVLHQDWLNGKEYKCKVSNKALPAPIEKTISKAKGQPREPQVYTLPPCRDELTKNQVSLWCLVKGFYPSDIAVEWESNGQPENNYKTTPPVLDSDGSFFLYSKLTVDKSRWQQGNVFSCSVMHEALHNHYTQKSLSLSPGK

SEQ ID NO: 84 - protein, 330 aa, Artificial Sequence
  synthetic construct
ASTKGPSVFPLAPSSKSTSGGTAALGCLVKDYFPEPVTVSWNSGALTSGVHTFPAVLQSSGLYSLSSVVTVPSSSLGTQTYICNVNHKPSNTKVDKKVEPKSCDKTHTCPPCPAPELLGGPSVFLFPPKPKDTLMISRTPEVTCVVVDVSHEDPEVKFNWYVDGVEVHNAKTKPREEQYNSTYRVVSVLTVLHQDWLNGKEYKCKVSNKALPAPIEKTISKAKGQPREPQVCTLPPSRDELTKNQVSLSCAVKGFYPSDIAVEWESNGQPENNYKTTPPVLDSDGSFFLVSKLTVDKSRWQQGNVFSCSVMHEALHNHYTQKSLSLSPGK

SEQ ID NO: 85 - protein, 330 aa, Artificial Sequence
  synthetic construct
ASTKGPSVFPLAPSSKSTSGGTAALGCLVKDYFPEPVTVSWNSGALTSGVHTFPAVLQSSGLYSLSSVVTVPSSSLGTQTYICNVNHKPSNTKVDKKVEPKSCDKTHTCPPCPAPELLGGPSVFLFPPKPKDTLMISRTPEVTCVVVDVSHEDPEVKFNWYVDGVEVHNAKTKPREEQYASTYRVVSVLTVLHQDWLNGKEYKCKVSNKALPAPIEKTISKAKGQPREPQVYTLPPCRDELTKNQVSLWCLVKGFYPSDIAVEWESNGQPENNYKTTPPVLDSDGSFFLYSKLTVDKSRWQQGNVFSCSVMHEALHNHYTQKSLSLSPGK

SEQ ID NO: 86 - protein, 330 aa, Artificial Sequence
  synthetic construct
ASTKGPSVFPLAPSSKSTSGGTAALGCLVKDYFPEPVTVSWNSGALTSGVHTFPAVLQSSGLYSLSSVVTVPSSSLGTQTYICNVNHKPSNTKVDKKVEPKSCDKTHTCPPCPAPELLGGPSVFLFPPKPKDTLMISRTPEVTCVVVDVSHEDPEVKFNWYVDGVEVHNAKTKPREEQYASTYRVVSVLTVLHQDWLNGKEYKCKVSNKALPAPIEKTISKAKGQPREPQVCTLPPSRDELTKNQVSLSCAVKGFYPSDIAVEWESNGQPENNYKTTPPVLDSDGSFFLVSKLTVDKSRWQQGNVFSCSVMHEALHNHYTQKSLSLSPGK

SEQ ID NO: 87 - DNA, 990 bp, Artificial Sequence
  synthetic construct
gcctccaccaagggcccctccgtgttccctctggccccctcttccaagagcaccagcggcggcaccgccgctctgggatgtctggtgaaggattactttcccgagcctgtgaccgtgagctggaactccggcgccctgacctccggcgtgcacacattccctgccgtgctgcagagcagcggcctgtactccctgagcagcgtggtgaccgtgcctagctccagcctgggcacccagacctacatctgtaacgtgaaccacaagccttccaacaccaaggtggacaagaaggtggagcctaagagctgtgacaagacccacacctgccctccttgtcctgcccctgagctgctgggcggcccatctgtgttcctgttccctcccaagcccaaggacaccctgatgatcagcagaacccccgaggtgacctgtgtggtggtggatgtgtcccacgaggaccctgaggtgaagtttaactggtacgtggatggcgtggaggtgcacaatgccaagaccaagcccagagaggagcagtacgcctccacctacagagtggtgtccgtgctgaccgtgctgcaccaggactggctgaatggcaaggagtacaagtgtaaggtgagcaacaaggccctgcccgcccctatcgagaagaccatcagcaaggccaagggccagcctagggagcctcaggtgtacaccctgcccccctgcagagacgagctgaccaagaatcaggtgagcctgtggtgcctggtgaagggcttctaccccagcgacatcgccgtggagtgggagtccaatggccagcctgagaacaattacaagaccaccccccctgtgctggatagcgatggcagcttctttctgtacagcaagctgaccgtggataagtccaggtggcagcagggcaatgtgtttagctgtagcgtgatgcacgaggccctgcacaatcactacacccagaagagcctgagcctgtcccccggcaag

SEQ ID NO: 88 - DNA, 990 bp, Artificial Sequence
  synthetic construct
gccagcaccaagggcccctccgtgttccctctggcccctagcagcaagtccaccagcggcggcaccgccgctctgggatgtctggtgaaggactactttcctgagcccgtgaccgtgtcctggaactccggcgccctgacctccggcgtgcacacattccccgccgtgctgcagtcctccggcctgtactccctgtccagcgtggtgaccgtgcctagctccagcctgggcacccagacctacatctgtaacgtgaaccacaagccctccaataccaaggtggataagaaggtggagcccaagtcctgcgacaagacccacacctgtcctccttgccccgcccccgagctgctgggaggaccttctgtgttcctgttccctcccaagcccaaggacaccctgatgatcagcagaacccctgaggtgacctgtgtggtggtggacgtgagccacgaggaccctgaggtgaagttcaactggtacgtggacggcgtggaggtgcacaatgccaagaccaagcccagagaggagcagtacgcctccacctacagagtggtgtccgtgctgaccgtgctgcaccaggattggctgaacggcaaggagtacaagtgcaaggtgtccaataaggccctgcccgcccccatcgagaagaccatctccaaggccaagggccagcccagagagcctcaggtgtgtaccctgcctccctccagggatgagctgaccaagaaccaggtgtccctgagctgcgccgtgaagggcttctaccccagcgatatcgccgtggagtgggagtccaacggccagcccgagaataattacaagaccaccccccccgtgctggacagcgacggatctttctttctggtgtccaagctgaccgtggataagtccaggtggcagcagggcaacgtgtttagctgtagcgtgatgcacgaggccctgcacaaccactacacccagaagtccctgtccctgagccccggcaag

SEQ ID NO: 89 - DNA, 321 bp, Artificial Sequence
  synthetic construct
cgtacggtggctgcaccatctgtcttcatcttcccgccatctgatgagcagttgaaatctggaactgcctctgttgtgtgcctgctgaataacttctatcccagagaggccaaagtacagtggaaggtggataacgccctccaatcgggtaactcccaggagagtgtcacagagcaggacagcaaggacagcacctacagcctcagcagcaccctgacgctgagcaaagcagactacgagaaacacaaagtctacgcctgcgaagtcacccatcagggcctgagctcgcccgtcacaaagagcttcaacaggggagagtgt

SEQ ID NO: 90 - protein, 19 aa, Artificial Sequence
  synthetic construct
MEFGLSWVFLVAILKGVQC

SEQ ID NO: 91 - protein, 22 aa, Artificial Sequence
  synthetic construct
MDMRVLAQLLGLLLLCFPGARC

SEQ ID NO: 92 - protein, 448 aa, Artificial Sequence
  synthetic construct
EVQLVESGGGLVQPGGSLRLSCAASGFTFSDSWIHWVRQAPGKGLEWVGWISPYGGSTYYADSYRSRFTISADTSKNTAYLQMNSLRAEDTAVYYCARRHWPGGFDYWGQGTLVTVSSASTKGPSVFPLAPSSKSTSGGTAALGCLVKDYFPEPVTVSWNSGALTSGVHTFPAVLQSSGLYSLSSVVTVPSSSLGTQTYICNVNHKPSNTKVDKKVEPKSCDKTHTCPPCPAPELLGGPSVFLFPPKPKDTLMISRTPEVTCVVVDVSHEDPEVKFNWYVDGVEVHNAKTKPREEQYASTYRVVSVLTVLHQDWLNGKEYKCKVSNKALPAPIEKTISKAKGQPREPQVYTLPPCRDELTKNQVSLWCLVKGFYPSDIAVEWESNGQPENNYKTTPPVLDSDGSFFLYSKLTVDKSRWQQGNVFSCSVMHEALHNHYTQKSLSLSPGK

SEQ ID NO: 93 - protein, 446 aa, Artificial Sequence
  synthetic construct
QVQLQESGPGLVKPSETLSLTCTVSGGSLDNYYWSWIRQPPGKGLEWIGYIYYSGNTNYNPSLKSRVTISVDTSKNQFSLKLSSVTAADTAVYYCARGGRFLERYWGQGTLVTVSSASTKGPSVFPLAPSSKSTSGGTAALGCLVKDYFPEPVTVSWNSGALTSGVHTFPAVLQSSGLYSLSSVVTVPSSSLGTQTYICNVNHKPSNTKVDKKVEPKSCDKTHTCPPCPAPELLGGPSVFLFPPKPKDTLMISRTPEVTCVVVDVSHEDPEVKFNWYVDGVEVHNAKTKPREEQYASTYRVVSVLTVLHQDWLNGKEYKCKVSNKALPAPIEKTISKAKGQPREPQVCTLPPSRDELTKNQVSLSCAVKGFYPSDIAVEWESNGQPENNYKTTPPVLDSDGSFFLVSKLTVDKSRWQQGNVFSCSVMHEALHNHYTQKSLSLSPGK

SEQ ID NO: 94 - protein, 448 aa, Artificial Sequence
  synthetic construct
EVQLVESGGGLVQPGGSLRLSCAASGFTFSDSWIHWVRQAPGKGLEWVGWISPYGGSTYYADSYRSRFTISADTSKNTAYLQMNSLRAEDTAVYYCARRHWPGGFDYWGQGTLVTVSSASTKGPSVFPLAPSSKSTSGGTAALGCLVKDYFPEPVTVSWNSGALTSGVHTFPAVLQSSGLYSLSSVVTVPSSSLGTQTYICNVNHKPSNTKVDKKVEPKSCDKTHTCPPCPAPELLGGPSVFLFPPKPKDTLMISRTPEVTCVVVDVSHEDPEVKFNWYVDGVEVHNAKTKPREEQYASTYRVVSVLTVLHQDWLNGKEYKCKVSNKALPAPIEKTISKAKGQPREPQVCTLPPSRDELTKNQVSLSCAVKGFYPSDIAVEWESNGQPENNYKTTPPVLDSDGSFFLVSKLTVDKSRWQQGNVFSCSVMHEALHNHYTQKSLSLSPGK

SEQ ID NO: 95 - protein, 446 aa, Artificial Sequence
  synthetic construct
QVQLQESGPGLVKPSETLSLTCTVSGGSLDNYYWSWIRQPPGKGLEWIGYIYYSGNTNYNPSLKSRVTISVDTSKNQFSLKLSSVTAADTAVYYCARGGRFLERYWGQGTLVTVSSASTKGPSVFPLAPSSKSTSGGTAALGCLVKDYFPEPVTVSWNSGALTSGVHTFPAVLQSSGLYSLSSVVTVPSSSLGTQTYICNVNHKPSNTKVDKKVEPKSCDKTHTCPPCPAPELLGGPSVFLFPPKPKDTLMISRTPEVTCVVVDVSHEDPEVKFNWYVDGVEVHNAKTKPREEQYASTYRVVSVLTVLHQDWLNGKEYKCKVSNKALPAPIEKTISKAKGQPREPQVYTLPPCRDELTKNQVSLWCLVKGFYPSDIAVEWESNGQPENNYKTTPPVLDSDGSFFLYSKLTVDKSRWQQGNVFSCSVMHEALHNHYTQKSLSLSPGK

SEQ ID NO: 96 - protein, 214 aa, Artificial Sequence
  synthetic construct
EIVLTQSPSSLSASVGDRVTITCLASQTIGTWLAWYQQKPGKSPQLLIYAASTLQSGVPSRFSGSGSGTDFTLTISSLQPEDVATYYCQQYYSTPRTFGQGTKVEIKRTVAAPSVFIFPPSDEQLKSGTASVVCLLNNFYPREAKVQWKVDNALQSGNSQESVTEQDSKDSTYSLSSTLTLSKADYEKHKVYACEVTHQGLSSPVTKSFNRGEC

SEQ ID NO: 97 - protein, 107 aa, Artificial Sequence
  synthetic construct
EIVLTQPPSSLSASVGDRVTIPCRASLSIGSFLNWYQQRPGEAPKLLIFAASSLRSGVPSRFSGSGSGTDFTLTISGLQPEDFATYYCQQTYTTPYTFGQGTKVDIK

SEQ ID NO: 98 - protein, 107 aa, Artificial Sequence
  synthetic construct
DIQMTQSPSSVSASVGDRVTISCRANQAIGTWLAWYQQKPGKAPKLLIYAASTLQSGVPSRFSGSGSGTEFTLTISSLQAEDVAVYYCQQYYTTPLTFGGGTKLEIK

SEQ ID NO: 99 - DNA, 1344 bp, Artificial Sequence
  synthetic construct
gaggtgcagctggtggaatccggcggagggctggtgcagccaggtggctctctgagactgagttgcgccgcttcaggattcaccttttccgactcttggattcactgggtgcgccaggcccccggaaagggactggagtgggtcggttggatttctccttacggagggagtacatactatgccgactcttataggtcgcgattcactatctccgctgatactagcaaaaacaccgcatatctgcagatgaactccctgagggcagaagacacagccgtctactattgtgcaaggcggcattggcccggtggctttgattactggggtcagggtaccctggtgaccgtgtcctccgcctccaccaagggcccctccgtgttccctctggccccctcttccaagagcaccagcggcggcaccgccgctctgggatgtctggtgaaggattactttcccgagcctgtgaccgtgagctggaactccggcgccctgacctccggcgtgcacacattccctgccgtgctgcagagcagcggcctgtactccctgagcagcgtggtgaccgtgcctagctccagcctgggcacccagacctacatctgtaacgtgaaccacaagccttccaacaccaaggtggacaagaaggtggagcctaagagctgtgacaagacccacacctgccctccttgtcctgcccctgagctgctgggcggcccatctgtgttcctgttccctcccaagcccaaggacaccctgatgatcagcagaacccccgaggtgacctgtgtggtggtggatgtgtcccacgaggaccctgaggtgaagtttaactggtacgtggatggcgtggaggtgcacaatgccaagaccaagcccagagaggagcagtacgcctccacctacagagtggtgtccgtgctgaccgtgctgcaccaggactggctgaatggcaaggagtacaagtgtaaggtgagcaacaaggccctgcccgcccctatcgagaagaccatcagcaaggccaagggccagcctagggagcctcaggtgtacaccctgcccccctgcagagacgagctgaccaagaatcaggtgagcctgtggtgcctggtgaagggcttctaccccagcgacatcgccgtggagtgggagtccaatggccagcctgagaacaattacaagaccaccccccctgtgctggatagcgatggcagcttctttctgtacagcaagctgaccgtggataagtccaggtggcagcagggcaatgtgtttagctgtagcgtgatgcacgaggccctgcacaatcactacacccagaagagcctgagcctgtcccccggcaag

SEQ ID NO: 100 - DNA, 1338 bp, Artificial Sequence
  synthetic construct
caggtgcagctgcaggagtccggccctggcctggtgaagccttccgagaccctgtccctgacctgtaccgtgagcggcggcagcctggataactattactggagctggatccggcagcctcctggcaagggcctggagtggatcggctacatctactattccggcaacaccaattacaacccttccctgaagagccgggtgaccatctccgtggacaccagcaagaaccagtttagcctgaagctgtcctccgtgaccgccgctgataccgccgtgtactactgtgccaggggcggccggttcctggagagatattggggccagggtaccctggtgaccgtgagcagcgccagcaccaagggcccctccgtgttccctctggcccctagcagcaagtccaccagcggcggcaccgccgctctgggatgtctggtgaaggactactttcctgagcccgtgaccgtgtcctggaactccggcgccctgacctccggcgtgcacacattccccgccgtgctgcagtcctccggcctgtactccctgtccagcgtggtgaccgtgcctagctccagcctgggcacccagacctacatctgtaacgtgaaccacaagccctccaataccaaggtggataagaaggtggagcccaagtcctgcgacaagacccacacctgtcctccttgccccgcccccgagctgctgggaggaccttctgtgttcctgttccctcccaagcccaaggacaccctgatgatcagcagaacccctgaggtgacctgtgtggtggtggacgtgagccacgaggaccctgaggtgaagttcaactggtacgtggacggcgtggaggtgcacaatgccaagaccaagcccagagaggagcagtacgcctccacctacagagtggtgtccgtgctgaccgtgctgcaccaggattggctgaacggcaaggagtacaagtgcaaggtgtccaataaggccctgcccgcccccatcgagaagaccatctccaaggccaagggccagcccagagagcctcaggtgtgtaccctgcctccctccagggatgagctgaccaagaaccaggtgtccctgagctgcgccgtgaagggcttctaccccagcgatatcgccgtggagtgggagtccaacggccagcccgagaataattacaagaccaccccccccgtgctggacagcgacggatctttctttctggtgtccaagctgaccgtggataagtccaggtggcagcagggcaacgtgtttagctgtagcgtgatgcacgaggccctgcacaaccactacacccagaagtccctgtccctgagccccggcaag

SEQ ID NO: 101 - DNA, 642 bp, Artificial Sequence
  synthetic construct
gaaattgtgctgactcagtctccatcctccctgtctgcatctgtaggagacagagtcaccatcacttgcctggcaagtcagaccattggtacatggttagcatggtatcagcagaaaccagggaaatctcctcagctcctgatctatgctgcatccactttgcaatcaggggtcccatctcggttcagtggcagtggatctgggacagatttcactctcaccatcagcagcctgcagcctgaagatgttgcaacttattactgtcagcaatattatagtactcctcggacgttcggccaagggaccaaggtggagattaaacgtacggtggctgcaccatctgtcttcatcttcccgccatctgatgagcagttgaaatctggaactgcctctgttgtgtgcctgctgaataacttctatcccagagaggccaaagtacagtggaaggtggataacgccctccaatcgggtaactcccaggagagtgtcacagagcaggacagcaaggacagcacctacagcctcagcagcaccctgacgctgagcaaagcagactacgagaaacacaaagtctacgcctgcgaagtcacccatcagggcctgagctcgcccgtcacaaagagcttcaacaggggagagtgt

SEQ ID NO: 102 - protein, 107 aa, Artificial Sequence
  synthetic construct
EIVLTQSPSSLSASVGDRVTIPCRASLSIGSFLNWYQQRPGEAPKLLIFAASSLRSGVPSRFSGSGSGTDFTLTISGLQPEDFATYYCQQTYTTPYTFGQGTKVDIK